European Patent Specification EP 3 845 666 B1, published January 7, 2026. Title: A METHOD OF DETECTING small RNA. Applicant: Xenohelix. Co., Ltd. The sequence listing filed with the application follows.

SEQUENCE LISTING (14 sequences)

SEQ ID NO: 1 - RNA, 22 nt, Artificial Sequence
  has-miR-21-5p
uagcuuaucagacugauguuga

SEQ ID NO: 2 - RNA, 22 nt, Artificial Sequence
  has-miR-210-3p
cugugcgugugacagcggcuga

SEQ ID NO: 3 - RNA, 22 nt, Artificial Sequence
  has-miR-486-5p
uccuguacugagcugccccgag

SEQ ID NO: 4 - DNA, 22 bp, Artificial Sequence
  sensing region of sensor DNA detecting for has-miR-486-5p
tcaacatcagtctgataagcta

SEQ ID NO: 5 - DNA, 22 bp, Artificial Sequence
  sensing region of sensor DNA detecting for has-miR-210-3p
tcagccgctgtcacacgcacag

SEQ ID NO: 6 - DNA, 22 bp, Artificial Sequence
  sensing region of sensor DNA detecting for has-miR-486-5p
ctcggggcagctcagtacagga

SEQ ID NO: 7 - DNA, 88 bp, Artificial Sequence
  module region of sensor DNA detecting for has-miR-21-5p
aacaataccacgaccaccgacaactacacgctacagtcgcatacgagatcgtgatgtgactggagttgcttggctctggtgtattggt

SEQ ID NO: 8 - DNA, 88 bp, Artificial Sequence
  module region of sensor DNA detecting for has-miR-210-3p
aacaataccacgaccaccgacaactacacgctacagtcgcatacgagatacatcggtgactggagttgcttggctctggtgtattggt

SEQ ID NO: 9 - DNA, 88 bp, Artificial Sequence
  module region of sensor DNA detecting for has-miR-486-5p
aacaataccacgaccaccgacaactacacgctacagtcgcatacgagatttaggcgtgactggagttgcttggctctggtgtattggt

SEQ ID NO: 10 - DNA, 6 bp, Artificial Sequence
  barcode region of sensor DNA detecting for has-miR-21-5p
cgtgat

SEQ ID NO: 11 - DNA, 6 bp, Artificial Sequence
  barcode region of sensor DNA detecting for has-miR-210-3p
acatcg

SEQ ID NO: 12 - DNA, 6 bp, Artificial Sequence
  barcode region of sensor DNA detecting for has-miR-486-5p
ttaggc

SEQ ID NO: 13 - DNA, 24 bp, Artificial Sequence
  Forward primer
aacaataccacgaccaccgacaac

SEQ ID NO: 14 - DNA, 24 bp, Artificial Sequence
  Reverse primer
accaatacaccagagccaagcaac